European Patent Specification EP 4 015 636 B1, published November 20, 2024. Title: 5' Triphosphate Oligonucleotides and Use Thereof. Applicant: Hartmann, Gunther. Application not yet assigned. The sequence listing filed with the application follows.

SEQUENCE LISTING (44 sequences)

SEQ ID NO: 1 - RNA, 23 nt, Artificial Sequence
  artificial sequence
gggggggggggaaaaaaaaaaaa

SEQ ID NO: 2 - RNA, 24 nt, Artificial Sequence
  artificial sequence
ggggcugacccugaaguucaucuu

SEQ ID NO: 3 - DNA, 20 bp, Artificial Sequence
  artificial sequence
gggggacgatcgtcgggggg

SEQ ID NO: 4 - RNA, 27 nt, Artificial Sequence
  artificial sequence
aagcugacccugaaguucaucugcacc

SEQ ID NO: 5 - RNA, 27 nt, Artificial Sequence
  artificial sequence
ggugcagaugaacuucagggucagcuu

SEQ ID NO: 6 - RNA, 29 nt, Artificial Sequence
  artificial sequence
gcugacccugaaguucaucugcaccacuu

SEQ ID NO: 7 - RNA, 27 nt, Artificial Sequence
  artificial sequence
guggugcagaugaacuucagggucagc

SEQ ID NO: 8 - RNA, 24 nt, Artificial Sequence
  artificial sequence
aacacacacacacacacacacuuu

SEQ ID NO: 9 - RNA, 24 nt, Artificial Sequence
  artificial sequence
gacacacacacacacacacacuuu

SEQ ID NO: 10 - RNA, 24 nt, Artificial Sequence
  artificial sequence
cacacacacacacacacacacuuu

SEQ ID NO: 11 - RNA, 24 nt, Artificial Sequence
  artificial sequence
uacacacacacacacacacacuuu

SEQ ID NO: 12 - RNA, 26 nt, Artificial Sequence
  artificial sequence
aaaguguguguguguguguguguugu

SEQ ID NO: 13 - RNA, 25 nt, Artificial Sequence
  artificial sequence
aaaguguguguguguguguguguug

SEQ ID NO: 14 - RNA, 26 nt, Artificial Sequence
  artificial sequence
aaaaaguguguguguguguguguguu

SEQ ID NO: 15 - RNA, 25 nt, Artificial Sequence
  artificial sequence
aaaaguguguguguguguguguguu

SEQ ID NO: 16 - RNA, 24 nt, Artificial Sequence
  artificial sequence
aaaguguguguguguguguguguu

SEQ ID NO: 17 - RNA, 23 nt, Artificial Sequence
  artificial sequence
aaguguguguguguguguguguu

SEQ ID NO: 18 - RNA, 21 nt, Artificial Sequence
  artificial sequence
guguguguguguguguguguu

SEQ ID NO: 19 - RNA, 20 nt, Artificial Sequence
  artificial sequence
uguguguguguguguguguu

SEQ ID NO: 20 - RNA, 19 nt, Artificial Sequence
  artificial sequence
guguguguguguguguguu

SEQ ID NO: 21 - RNA, 17 nt, Artificial Sequence
  artificial sequence
guguguguguguguguu

SEQ ID NO: 22 - RNA, 15 nt, Artificial Sequence
  artificial sequence
guguguguguguguu

SEQ ID NO: 23 - RNA, 13 nt, Artificial Sequence
  artificial sequence
guguguguguguu

SEQ ID NO: 24 - RNA, 26 nt, Artificial Sequence
  artificial sequence
aaagugugugugugugugugugucgu

SEQ ID NO: 25 - RNA, 25 nt, Artificial Sequence
  artificial sequence
aaagugugugugugugugugugucg

SEQ ID NO: 26 - RNA, 26 nt, Artificial Sequence
  artificial sequence
aaaaaguguguguguguguguguguc

SEQ ID NO: 27 - RNA, 25 nt, Artificial Sequence
  artificial sequence
aaaaguguguguguguguguguguc

SEQ ID NO: 28 - RNA, 24 nt, Artificial Sequence
  artificial sequence
aaaguguguguguguguguguguc

SEQ ID NO: 29 - RNA, 23 nt, Artificial Sequence
  artificial sequence
aaguguguguguguguguguguc

SEQ ID NO: 30 - RNA, 21 nt, Artificial Sequence
  artificial sequence
guguguguguguguguguguc

SEQ ID NO: 31 - RNA, 20 nt, Artificial Sequence
  artificial sequence
uguguguguguguguguguc

SEQ ID NO: 32 - RNA, 19 nt, Artificial Sequence
  artificial sequence
guguguguguguguguguc

SEQ ID NO: 33 - RNA, 17 nt, Artificial Sequence
  artificial sequence
guguguguguguguguc

SEQ ID NO: 34 - RNA, 15 nt, Artificial Sequence
  artificial sequence
guguguguguguguc

SEQ ID NO: 35 - RNA, 13 nt, Artificial Sequence
  artificial sequence
guguguguguguc

SEQ ID NO: 36 - RNA, 26 nt, Artificial Sequence
  artificial sequence
aaaguguguguguguguguguguggu

SEQ ID NO: 37 - RNA, 24 nt, Artificial Sequence
  artificial sequence
aaagugugugugugugugugugug

SEQ ID NO: 38 - RNA, 26 nt, Artificial Sequence
  artificial sequence
aaaguguguguguguguguguguagu

SEQ ID NO: 39 - RNA, 24 nt, Artificial Sequence
  artificial sequence
aaagugugugugugugugugugua

SEQ ID NO: 40 - RNA, 23 nt, Artificial Sequence
  artificial sequence
aaagugugugugugugugugugu

SEQ ID NO: 41 - RNA, 21 nt, Artificial Sequence
  artificial sequence
aaagugugugugugugugugu

SEQ ID NO: 42 - RNA, 19 nt, Artificial Sequence
  artificial sequence
aaagugugugugugugugu

SEQ ID NO: 43 - RNA, 30 nt, Artificial Sequence
  artificial sequence
gacgacgacgacgacgacgacgacgacgac

SEQ ID NO: 44 - RNA, 24 nt, Artificial Sequence
  artificial sequence
gacacacacacacacacacacaca